European Patent Application EP 4 349 862 A1, published April 10, 2024. Title: ANTI-HUMAN INTERFERON α RECEPTOR 1 MONOCLONAL ANTIBODY AND APPLICATION THEREOF. Applicant: Qyuns Therapeutics Co., Ltd. The sequence listing filed with the application follows.

SEQUENCE LISTING (11 sequences)

SEQ ID NO: 1 - protein, 5 aa, Artificial Sequence
  Artificial
SYYMT

SEQ ID NO: 2 - protein, 16 aa, Artificial Sequence
  Artificial
VINVYGGTYYASWAKG

SEQ ID NO: 3 - protein, 11 aa, Artificial Sequence
  Artificial
EDVAVYMAIDL

SEQ ID NO: 4 - protein, 11 aa, Artificial Sequence
  Artificial
QASQSISNQLS

SEQ ID NO: 5 - protein, 7 aa, Artificial Sequence
  Artificial
DASSLAS

SEQ ID NO: 6 - protein, 13 aa, Artificial Sequence
  Artificial
LGIYGDGADDGIA

SEQ ID NO: 7 - protein, 119 aa, Artificial Sequence
  Artificial
EVQLVESGGGLVQPGGSLRLSCAASGFSLSSYYMTWVRQAPGKGLEWVSVINVYGGTYYASWAKGRFTISRDNSKNTLYLQMNSLRAEDTAVYYCAREDVAVYMAIDLWGQGTLVTVSS

SEQ ID NO: 8 - protein, 111 aa, Artificial Sequence
  Artificial
AIQMTQSPSSLSASVGDRVTITCQASQSISNQLSWYQQKPGKAPKLLIYDASSLASGVPSRFSGSRSGTKFTLTISSLQPEDFATYYCLGIYGDGADDGIAFGGGTKVEIK

SEQ ID NO: 9 - protein, 436 aa, Artificial Sequence
  Artificial
MMVVLLGATTLVLVAVAPWVLSAAAGGKNLKSPQKVEVDIIDDNFILRWNRSDESVGNVTFSFDYQKTGMDNWIKLSGCQNITSTKCNFSSLKLNVYEEIKLRIRAEKENTSSWYEVDSFTPFRKAQIGPPEVHLEAEDKAIVIHISPGTKDSVMWALDGLSFTYSLVIWKNSSGVEERIENIYSRHKIYKLSPETTYCLKVKAALLTSWKIGVYSPVHCIKTTVENELPPPENIEVSVQNQNYVLKWDYTYANMTFQVQWLHAFLKRNPGNHLYKWKQIPDCENVKTTQCVFPQNVFQKGIYLLRVQASDGNNTSFWSEEIKFDTEIQAFLLPPVFNIRSLSDSFHIYIGAPKQSGNTPVIQDYPLIYEIIFWENTSNAERKIIEKKTDVTVPNLKPLTVYCVKARAHTMDEKLNKSSVFSDAVCEKTKPGNTSK

SEQ ID NO: 10 - protein, 446 aa, Artificial Sequence
  Artificial
EVQLVESGGGLVQPGGSLRLSCAASGFSLSSYYMTWVRQAPGKGLEWVSVINVYGGTYYASWAKGRFTISRDNSKNTLYLQMNSLRAEDTAVYYCAREDVAVYMAIDLWGQGTLVTVSSASTKGPSVFPLAPCSRSTSESTAALGCLVKDYFPEPVTVSWNSGALTSGVHTFPAVLQSSGLYSLSSVVTVPSSSLGTKTYTCNVDHKPSNTKVDKRVESKYGPPCPPCPAPEFLGGPSVFLFPPKPKDTLMISRTPEVTCVVVDVSQEDPEVQFNWYVDGVEVHNAKTKPREEQFNSTYRVVSVLTVLHQDWLNGKEYKCKVSNKGLPSSIEKTISKAKGQPREPQVYTLPPSQEEMTKNQVSLTCLVKGFYPSDIAVEWESNGQPENNYKTTPPVLDSDGSFFLYSRLTVDKSRWQEGNVFSCSVMHEALHNHYTQKSLSLSLGK

SEQ ID NO: 11 - protein, 218 aa, Artificial Sequence
  Artificial
AIQMTQSPSSLSASVGDRVTITCQASQSISNQLSWYQQKPGKAPKLLIYDASSLASGVPSRFSGSRSGTKFTLTISSLQPEDFATYYCLGIYGDGADDGIAFGGGTKVEIKRTVAAPSVFIFPPSDEQLKSGTASVVCLLNNFYPREAKVQWKVDNALQSGNSQESVTEQDSKDSTYSLSSTLTLSKADYEKHKVYACEVTHQGLSSPVTKSFNRGEC